European Patent Application EP 4 509 518 A1, published February 19, 2025. Title: FUSION TYPE ADENO-ASSOCIATED VIRUS AND USE THEREOF. Applicant: Starrygene Therapeutics Co., Ltd. The sequence listing filed with the application follows.

SEQUENCE LISTING (9 sequences)

SEQ ID NO: 1 - DNA, 2211 bp, synthetic construct
  source 1..2211: mol_type = other DNA
atggctgccgatggttatcttccagattggctcgaggacaacctctctgagggcattcgcgagtggtgggacttgaaacctggagccccgaagcccaaagccaaccagcaaaagcaggacgacggccggggtctggtgcttcctggctacaagtacctcggacccttcaacggactcgacaagggggagcccgtcaacgcggcggacgcagcggccctcgagcacgacaaggcctacgaccagcagctcaaagcgggtgacaatccgtacctgcggtataaccacgccgacgccgagtttcaggagcgtctgcaagaagatacgtcttttgggggcaacctcgggcgagcagtcttccaggccaagaagcgggttctcgaacctctcggtctggttgaggaaggcgctaagacggctcctggaaagaaacgtccggtagagcagtcgccacaagagccagactcctcctcgggcatcggcaagacaggccagcagcccgctaaaaagagactcaattttggtcagactggcgactcagagtcagtccccgatccacaacctctcggagaacctccagcaacccccgctgctgtgggacctactacaatggcttcaggcggtggcgcaccaatggcagacaataacgaaggcgccgacggagtgggtaatgcctcaggaaattggcattgcgattccacatggctgggcgacagagtcatcaccaccagcacccgcacctgggccctgcccacctacaacaatcacctctacaagcaaatctccagtgaaactgcaggtagtaccaacgacaacacctacttcggctacagcaccccctgggggtattttgactttaacagattccactgccacttctcaccacgtgactggcagcgactcatcaacaacaactggggattccggcccaagaagctgcggttcaagctcttcaacatccaggtcaaggaggtcacgcagaatgacggtacgacgacgattgccaataaccttaccagcacggttcaggtgtttactgactcggagtaccagctcccgtacgtcctcggctcggcgcatcaaggatgcctcccgccgttcccagcagacgtcttcatggtgccacagtatggatacctcaccctgaacaacgggagtcaggcagtaggacgctcttcattttactgcctggaatatttcccatcgcagatgctgagaacgggcaataactttaccttcagctacacctttgaggaagtgcctttccacagcagctacgcgcacagccagatcctggaccggctgatgaatcctctcatcgaccaatacctgtattacctgaacagaactcaaaatcagtccggaagtgcccaaaacaaggacttgctgtttagccgtgggtctccagctggcatgtctgttcagcccaaaaactggctacctggaccctgttatcggcagcagcgcgtttctaaaacaaaaacagacaacaacaacagcaattttacctggactggtgcttcaaaatataacctcaatgggcgtgaatccatcatcaaccctggcactgctatggcctcacacaaagacgacgaagacaagttctttcccatgagcggtgtcatgatttttggaaaagagagcgccggagcttcaaacactgcattggacaatgtcatgatcacagacgaagaggaaatcaaagccactaaccccgtggccaccgaaagatttgggactgtggcagtcaatctccagagcagcagcacagaccctgcgaccggagatgtgcatgttatgggagccttacctggaatggtgtggcaagacagagacgtatacctgcagggacccatttgggccaagattcctcacaccgatggacactttcatccttctccactgatgggaggttttgggctcaaacacccgcctcctcagatcctcatcaaaaacacgcctgttcctgcgaatcctccggcggagttttcagctacaaagtttgcttcattcatcacccaatactccacaggacaagtgagtgtggaaattgaatgggagctgcagaaagaaaacagcaagcgctggaatcccgaagtgcagtacacatccaattatgcaaaatctgccaacgttgattttactgtggacaacaatggactttatactgagcctcgccccattggcacccgttaccttacccgtcccctgtaa

SEQ ID NO: 2 - protein, 736 aa, synthetic construct
MAADGYLPDWLEDNLSEGIREWWDLKPGAPKPKANQQKQDDGRGLVLPGYKYLGPFNGLDKGEPVNAADAAALEHDKAYDQQLKAGDNPYLRYNHADAEFQERLQEDTSFGGNLGRAVFQAKKRVLEPLGLVEEGAKTAPGKKRPVEQSPQEPDSSSGIGKTGQQPAKKRLNFGQTGDSESVPDPQPLGEPPATPAAVGPTTMASGGGAPMADNNEGADGVGNASGNWHCDSTWLGDRVITTSTRTWALPTYNNHLYKQISSETAGSTNDNTYFGYSTPWGYFDFNRFHCHFSPRDWQRLINNNWGFRPKKLRFKLFNIQVKEVTQNDGTTTIANNLTSTVQVFTDSEYQLPYVLGSAHQGCLPPFPADVFMVPQYGYLTLNNGSQAVGRSSFYCLEYFPSQMLRTGNNFTFSYTFEEVPFHSSYAHSQILDRLMNPLIDQYLYYLNRTQNQSGSAQNKDLLFSRGSPAGMSVQPKNWLPGPCYRQQRVSKTKTDNNNSNFTWTGASKYNLNGRESIINPGTAMASHKDDEDKFFPMSGVMIFGKESAGASNTALDNVMITDEEEIKATNPVATERFGTVAVNLQSSSTDPATGDVHVMGALPGMVWQDRDVYLQGPIWAKIPHTDGHFHPSPLMGGFGLKHPPPQILIKNTPVPANPPAEFSATKFASFITQYSTGQVSVEIEWELQKENSKRWNPEVQYTSNYAKSANVDFTVDNNGLYTEPRPIGTRYLTRPL

SEQ ID NO: 3 - protein, 262 aa, synthetic construct
MAADGYLPDWLEDNLSEGIREWWDLKPGAPKPKANQQKQDDGRGLVLPGYKYLGPFNGLDKGEPVNAADAAALEHDKAYDQQLKAGDNPYLRYNHADAEFQERLQEDTSFGGNLGRAVFQAKKRVLEPLGLVEEGAKTAPGKKRPVEQSPQEPDSSSGIGKTGQQPAKKRLNFGQTGDSESVPDPQPLGEPPATPAAVGPTTMASGGGAPMADNNEGADGVGNASGNWHCDSTWLGDRVITTSTRTWALPTYNNHLYKQISS

SEQ ID NO: 4 - protein, 63 aa, synthetic construct
ETAGSTNDNTYFGYSTPWGYFDFNRFHCHFSPRDWQRLINNNWGFRPKKLRFKLFNIQVKEVT

SEQ ID NO: 5 - protein, 92 aa, synthetic construct
QNDGTTTIANNLTSTVQVFTDSEYQLPYVLGSAHQGCLPPFPADVFMVPQYGYLTLNNGSQAVGRSSFYCLEYFPSQMLRTGNNFTFSYTFE

SEQ ID NO: 6 - protein, 166 aa, synthetic construct
EVPFHSSYAHSQILDRLMNPLIDQYLYYLNRTQNQSGSAQNKDLLFSRGSPAGMSVQPKNWLPGPCYRQQRVSKTKTDNNNSNFTWTGASKYNLNGRESIINPGTAMASHKDDEDKFFPMSGVMIFGKESAGASNTALDNVMITDEEEIKATNPVATERFGTVAVN

SEQ ID NO: 7 - protein, 153 aa, synthetic construct
LQSSSTDPATGDVHVMGALPGMVWQDRDVYLQGPIWAKIPHTDGHFHPSPLMGGFGLKHPPPQILIKNTPVPANPPAEFSATKFASFITQYSTGQVSVEIEWELQKENSKRWNPEVQYTSNYAKSANVDFTVDNNGLYTEPRPIGTRYLTRPL

SEQ ID NO: 8 - DNA, 23 bp, synthetic construct
  source 1..23: mol_type = other DNA
gtcaggcaacgtggcgtggtgtg

SEQ ID NO: 9 - DNA, 21 bp, synthetic construct
  source 1..21: mol_type = other DNA
ggcgatgagttccgccgtggc